European Patent Specification EP 3 501 536 B1, published December 24, 2025. Title: Treatment of Ocular Disease. Applicant: Aerpio Therapeutics, Inc. The sequence listing filed with the application follows.

SEQUENCE LISTING (7 sequences)

SEQ ID NO: 1 - DNA, 6045 bp, Homo sapiens
atgctgagccatggagccgggttggccttgtggatcacactgagcctgctgcagactggactggcggagccagagagatgtaacttcaccctggcggagtccaaggcctccagccattctgtgtctatccagtggagaattttgggctcaccctgtaactttagcctcatctatagcagtgacaccctgggggccgcgttgtgccctacctttcggatagacaacaccacatacggatgtaaccttcaagatttacaagcaggaaccatctataacttcaagattatttctctggatgaagagagaactgtggtcttgcaaacagatcctttacctcctgctaggtttggagtcagtaaagagaagacgacttcaaccggcttgcatgtttggtggactccttcttccggaaaagtcacctcatatgaggtgcaattatttgatgaaaataaccaaaagatacagggggttcaaattcaagaaagtacttcatggaatgaatacacttttttcaatctcactgctggtagtaaatacaatattgccatcacagctgtttctggaggaaaacgttctttttcagtttataccaatggatcaacagtgccatctccagtgaaagatattggtatttccacaaaagccaattctctcctgatttcctggtcccatggttctgggaatgtggaacgataccggctgatgctaatggataaagggatcctagttcatggcggtgttgtggacaaacatgctacttcctatgcttttcacgggctgtcccctggctacctctacaacctcactgttatgactgaggctgcagggctgcaaaactacaggtggaaactagtcaggacagcccccatggaagtctcaaatctgaaggtgacaaatgatggcagtttgacctctctaaaagtcaaatggcaaagacctcctggaaatgtggattcttacaatatcaccctgtctcacaaagggaccatcaaggaatccagagtattagcaccttggattactgaaactcactttaaagagttagtccccggtcgactttatcaagttactgtcagctgtgtctctggtgaactgtctgctcagaagatggcagtgggcagaacatttccagacaaagttgcaaacctggaggcaaacaataatggcaggatgaggtctcttgtagtgagctggtcgccccctgctggagactgggagcagtatcggatcctactcttcaatgattctgtggtgctgctcaacatcactgtgggaaaggaagaaacacagtatgtcatggatgacacggggctcgtaccgggaagacagtatgaggtggaagtcattgttgagagtggaaatttgaagaattctgagcgttgccaaggcaggacagtccccctggctgtcctccagcttcgtgtcaaacatgccaatgaaacctcactgagtatcatgtggcagacccctgtagcagaatgggagaaatacatcatttccctagctgacagagacctcttactgatccacaagtcactctccaaagatgccaaagaattcacttttactgacctggtgcctggacgaaaatacatggctacagtcaccagtattagtggagacttaaaaaattcctcttcagtaaaaggaagaacagtgcctgcccaagtgactgacttgcatgtggccaaccaaggaatgaccagtagtctgtttactaactggacccaggcacaaggagacgtagaattttaccaagtcttactgatccatgaaaatgtggtcattaaaaatgaaagcatctccagtgagaccagcagatacagcttccactctctcaagtccggcagcctgtactccgtggtggtaacaacagtgagtggagggatctcttcccgacaagtggttgtggagggaagaacagtcccttccagtgtgagtggagtaacggtgaacaattccggtcgtaatgactacctcagcgtttcctggctcgtggcgcccggagatgtggataactatgaggtaacattgtctcatgacggcaaggtggttcagtcccttgtcattgccaagtctgtcagagaatgttccttcagctccctcaccccaggccgcctctacaccgtgaccataactacaaggagtggcaagtatgaaaatcactccttcagccaagagcggacagtgcctgacaaagtccagggagtcagtgttagcaactcagccaggagtgactatttaagggtatcctgggtgcatgccactggagactttgatcactatgaagtcaccattaaaaacaaaaacaacttcattcaaactaaaagcattcccaagtcagaaaacgaatgtgtatttgttcagctagtccctggacggttgtacagtgtcactgttactacaaaaagtggacaatatgaagccaatgaacaagggaatgggagaacaattccagagcctgttaaggatctaacattgcgcaacaggagcactgaggacttgcatgtgacttggtcaggagctaatggggatgtcgaccaatatgagatccagctgctcttcaatgacatgaaagtatttcctccttttcaccttgtaaataccgcaaccgagtatcgatttacttccctaacaccaggccgccaatacaaaattcttgtcttgacgattagcggggatgtacagcagtcagccttcattgagggcttcacagttcctagtgctgtcaaaaatattcacatttctcccaatggagcaacagatagcctgacggtgaactggactcctggtgggggagacgttgattcctacacggtgtcggcattcaggcacagtcaaaaggttgactctcagactattcccaagcacgtctttgagcacacgttccacagactggaggccggggagcagtaccagatcatgattgcctcagtcagcgggtccctgaagaatcagataaatgtggttgggcggacagttccagcatctgtccaaggagtaattgcagacaatgcatacagcagttattccttaatagtaagttggcaaaaagctgctggtgtggcagaaagatatgatatcctgcttctaactgaaaatggaatccttctgcgcaacacatcagagccagccaccactaagcaacacaaatttgaagatctaacaccaggcaagaaatacaagatacagatcctaactgtcagtggaggcctctttagcaaggaagcccagactgaaggccgaacagtcccagcagctgtcaccgacctgaggatcacagagaactccaccaggcacctgtccttccgctggaccgcctcagagggggagctcagctggtacaacatctttttgtacaacccagatgggaatctccaggagagagctcaagttgacccactagtccagagcttctctttccagaacttgctacaaggcagaatgtacaagatggtgattgtaactcacagtggggagctgtctaatgagtctttcatatttggtagaacagtcccagcctctgtgagtcatctcagggggtccaatcggaacacgacagacagcctttggttcaactggagtccagcctctggggactttgacttttatgagctgattctctataatcccaatggcacaaagaaggaaaactggaaagacaaggacctgacggagtggcggtttcaaggccttgttcctggaaggaagtacgtgctgtgggtggtaactcacagtggagatctcagcaataaagtcacagcggagagcagaacagctccaagtcctcccagtcttatgtcatttgctgacattgcaaacacatccttggccatcacgtggaaagggcccccagactggacagactacaacgactttgagctgcagtggttgcccagagatgcacttactgtcttcaacccctacaacaacagaaaatcagaaggacgcattgtgtatggtcttcgtccagggagatcctatcaattcaacgtcaagactgtcagtggtgattcctggaaaacttacagcaaaccaatttttggatctgtgaggacaaagcctgacaagatacaaaacctgcattgccggcctcagaactccacggccattgcctgttcttggatccctcctgattctgactttgatggttatagtattgaatgccggaaaatggacacccaagaagttgagttttccagaaagctggagaaagaaaaatctctgctcaacatcatgatgctagtgccccataagaggtacctggtgtccatcaaagtgcagtcggccggcatgaccagcgaggtggttgaagacagcactatcacaatgatagaccgcccccctcctccacccccacacattcgtgtgaatgaaaaggatgtgctaattagcaagtcttccatcaactttactgtcaactgcagctggttcagcgacaccaatggagctgtgaaatacttcacagtggtggtgagagaggctgatggcagtgatgagctgaagccagaacagcagcaccctctcccttcctacctggagtacaggcacaatgcctccattcgggtgtatcagactaattattttgccagcaaatgtgccgaaaatcctaacagcaactccaagagttttaacattaagcttggagcagagatggagagcttaggtggaaaacgcgatcccactcagcaaaaattctgtgatggaccactgaagccacacactgcctacagaatcagcattcgagcttttacacagctctttgatgaggacctgaaggaattcacaaagccactctattcagacacatttttttctttacccatcactactgaatcagagcccttgtttggagctattgaaggtgtgagtgctggtctgtttttaattggcatgctagtggctgttgttgccttattgatctgcagacagaaagtgagccatggtcgagaaagaccctctgcccgtctgagcattcgtagggatcgaccattatctgtccacttaaacctgggccagaaaggtaaccggaaaacttcttgtccaataaaaataaatcagtttgaagggcatttcatgaagctacaggctgactccaactaccttctatccaaggaatacgaggagttaaaagacgtgggccgaaaccagtcatgtgacattgcactcttgccggagaatagagggaaaaatcgatacaacaatatattgccctatgatgccacgcgagtgaagctctccaatgtagatgatgatccttgctctgactacatcaatgccagctacatccctggcaacaacttcagaagagaatacattgtcactcagggaccgcttcctggcaccaaggatgacttctggaaaatggtgtgggaacaaaacgttcacaacatcgtcatggtgacccagtgtgttgagaagggccgagtaaagtgtgaccattactggccagcggaccaggattccctctactatggggacctcatcctgcagatgctctcagagtccgtcctgcctgagtggaccatccgggagtttaagatatgcggtgaggaacagcttgatgcacacagactcatccgccactttcactatacggtgtggccagaccatggagtcccagaaaccacccagtctctgatccagtttgtgagaactgtcagggactacatcaacagaagcccgggtgctgggcccactgtggtgcactgcagtgctggtgtgggtaggactggaacctttattgcattggaccgaatcctccagcagttagactccaaagactctgtggacatttatggagcagtgcacgacctaagacttcacagggttcacatggtccagactgagtgtcagtatgtctacctacatcagtgtgtaagagatgtcctcagagcaagaaagctacggagtgaacaagaaaaccccttgtttccaatctatgaaaatgtgaatccagagtatcacagagatccagtctattcaaggcattgagaatgtacctgaagagctcctggataaaaattattcactgtgtgatttgtt

SEQ ID NO: 2 - protein, 1997 aa, Homo sapiens
MLSHGAGLALWITLSLLQTGLAEPERCNFTLAESKASSHSVSIQWRILGSPCNFSLIYSSDTLGAALCPTFRIDNTTYGCNLQDLQAGTIYNFRIISLDEERTVVLQTDPLPPARFGVSKEKTTSTSLHVWWTPSSGKVTSYEVQLFDENNQKIQGVQIQESTSWNEYTFFNLTAGSKYNIAITAVSGGKRSFSVYTNGSTVPSPVKDIGISTKANSLLISWSHGSGNVERYRLMLMDKGILVHGGVVDKHATSYAFHGLTPGYLYNLTVMTEAAGLQNYRWKLVRTAPMEVSNLKVTNDGSLTSLKVKWQRPPGNVDSYNITLSHKGTIKESRVLAPWITETHFKELVPGRLYQVTVSCVSGELSAQKMAVGRTFPDKVANLEANNNGRMRSLVVSWSPPAGDWEQYRILLFNDSVVLLNITVGKEETQYVMDDTGLVPGRQYEVEVIVESGNLKNSERCQGRTVPLAVLQLRVKHANETSLSIMWQTPVAEWEKYIISLADRDLLLIHKSLSKDAKEFTFTDLVPGRKYMATVTSISGDLKNSSSVKGRTVPAQVTDLHVANQGMTSSLFTNWTQAQGDVEFYQVLLIHENVVIKNESISSETSRYSFHSLKSGSLYSVVVTTVSGGISSRQVVVEGRTVPSSVSGVTVNNSGRNDYLSVSWLLAPGDVDNYEVTLSHDGKVVQSLVIAKSVRECSFSSLTPGRLYTVTITTRSGKYENHSFSQERTVPDKVQGVSVSNSARSDYLRVSWVHATGDFDHYEVTIKNKNNFIQTKSIPKSENECVFVQLVPGRLYSVTVTTKSGQYEANEQGNGRTIPEPVKDLTLRNRSTEDLHVTWSGANGDVDQYEIQLLFNDMKVFPPFHLVNTATEYRFTSLTPGRQYKILVLTISGDVQQSAFIEGFTVPSAVKNIHISPNGATDSLTVNWTPGGGDVDSYTVSAFRHSQKVDSQTIPKHVFEHTFHRLEAGEQYQIMIASVSGSLKNQINVVGRTVPASVQGVIADNAYSSYSLIVSWQKAAGVAERYDILLLTENGILLRNTSEPATTKQHKFEDLTPGKKYKIQILTVSGGLFSKEAQTEGRTVPAAVTDLRITENSTRHLSFRWTASEGELSWYNIFLYNPDGNLQERAQVDPLVQSFSFQNLLQGRMYKMVIVTHSGELSNESFIFGRTVPASVSHLRGSNRNTTDSLWFNWSPASGDFDFYELILYNPNGTKKENWKDKDLTEWRFQGLVPGRKYVLWVVTHSGDLSNKVTAESRTAPSPPSLMSFADIANTSLAITWKGPPDWTDYNDFELQWLPRDALTVFNPYNNRKSEGRIVYGLRPGRSYQFNVKTVSGDSWKTYSKPIFGSVRTKPDKIQNLHCRPQNSTAIACSWIPPDSDFDGYSIECRKMDTQEVEFSRKLEKEKSLLNIMMLVPHKRYLVSIKVQSAGMTSEVVEDSTITMIDRPPPPPPHIRVNEKDVLISKSSINFTVNCSWFSDTNGAVKYFTVVVREADGNDELKPEQQHPLPSYLEYRHNASIRVYQTNYFASKCAENPNSNSKSFNIKLGAEMESLGGKCDPTQQKFCDGPLKPHTAYRISIRAFTQLFDEDLKEFTKPLYSDTFFSLPITTESEPLFGAIEGVSAGLFLIGMLVAVVALLICRQKVSHGRERPSARLSIRRDRPLSVHLNLGQKGNRKTSCPIKINQFEGHFMKLQADSNYLLSKEYEELKDVGRNQSCDIALLPENRGKNRYNNILPYDATRVKLSNVDDDPCSDYINASYIPGNNFRREYIVTQGPLPGTKDDFWKMVWEQNVHNIVMVTQCVEKGRVKCDHYWPADQDSLYYGDLILQMLSESVLPEWTIREFKICGEEQLDAHRLIRHFHYTVWPDHGVPETTQSLIQFVRTVRDYINRSPGAGPTVVHCSAGVGRTGTFIALDRILQQLDSKDSVDIYGAVHDLRLHRVHMVQTECQYVYLHQCVRDVLRARKLRSEQENPLFPIYENVNPEYHRDPVYSRH

SEQ ID NO: 3 - protein, 1631 aa, Homo sapiens
MLSHGAGLALWITLSLLQTGLAEPERCNFTLAESKASSHSVSIQWRILGSPCNFSLIYSSDTLGAALCPTFRIDNTTYGCNLQDLQAGTIYNFRIISLDEERTVVLQTDPLPPARFGVSKEKTTSTSLHVWWTPSSGKVTSYEVQLFDENNQKIQGVQIQESTSWNEYTFFNLTAGSKYNIAITAVSGGKRSFSVYTNGSTVPSPVKDIGISTKANSLLISWSHGSGNVERYRLMLMDKGILVHGGVVDKHATSYAFHGLTPGYLYNLTVMTEAAGLQNYRWKLVRTAPMEVSNLKVTNDGSLTSLKVKWQRPPGNVDSYNITLSHKGTIKESRVLAPWITETHFKELVPGRLYQVTVSCVSGELSAQKMAVGRTFPDKVANLEANNNGRMRSLVVSWSPPAGDWEQYRILLFNDSVVLLNITVGKEETQYVMDDTGLVPGRQYEVEVIVESGNLKNSERCQGRTVPLAVLQLRVKHANETSLSIMWQTPVAEWEKYIISLADRDLLLIHKSLSKDAKEFTFTDLVPGRKYMATVTSISGDLKNSSSVKGRTVPAQVTDLHVANQGMTSSLFTNWTQAQGDVEFYQVLLIHENVVIKNESISSETSRYSFHSLKSGSLYSVVVTTVSGGISSRQVVVEGRTVPSSVSGVTVNNSGRNDYLSVSWLLAPGDVDNYEVTLSHDGKVVQSLVIAKSVRECSFSSLTPGRLYTVTITTRSGKYENHSFSQERTVPDKVQGVSVSNSARSDYLRVSWVHATGDFDHYEVTIKNKNNFIQTKSIPKSENECVFVQLVPGRLYSVTVTTKSGQYEANEQGNGRTIPEPVKDLTLRNRSTEDLHVTWSGANGDVDQYEIQLLFNDMKVFPPFHLVNTATEYRFTSLTPGRQYKILVLTISGDVQQSAFIEGFTVPSAVKNIHISPNGATDSLTVNWTPGGGDVDSYTVSAFRHSQKVDSQTIPKHVFEHTFHRLEAGEQYQIMIASVSGSLKNQINVVGRTVPASVQGVIADNAYSSYSLIVSWQKAAGVAERYDILLLTENGILLRNTSEPATTKQHKFEDLTPGKKYKIQILTVSGGLFSKEAQTEGRTVPAAVTDLRITENSTRHLSFRWTASEGELSWYNIFLYNPDGNLQERAQVDPLVQSFSFQNLLQGRMYKMVIVTHSGELSNESFIFGRTVPASVSHLRGSNRNTTDSLWFNWSPASGDFDFYELILYNPNGTKKENWKDKDLTEWRFQGLVPGRKYVLWVVTHSGDLSNKVTAESRTAPSPPSLMSFADIANTSLAITWKGPPDWTDYNDFELQWLPRDALTVFNPYNNRKSEGRIVYGLRPGRSYQFNVKTVSGDSWKTYSKPIFGSVRTKPDKIQNLHCRPQNSTAIACSWIPPDSDFDGYSIECRKMDTQEVEFSRKLEKEKSLLNIMMLVPHKRYLVSIKVQSAGMTSEVVEDSTITMIDRPPPPPPHIRVNEKDVLISKSSINFTVNCSWFSDTNGAVKYFTVVVREADGNDELKPEQQHPLPSYLEYRHNASIRVYQTNYFASKCAENPNSNSKSFNIKLGAEMESLGGKCDPTQQKFCDGPLKPHTAYRISIRAFTQLFDEDLKEFTKPLYSDTFFSLPITTESEPLFGAIERGRHHHHHHG

SEQ ID NO: 4 - protein, 1621 aa, Homo sapiens
MLSHGAGLALWITLSLLQTGLAEPERCNFTLAESKASSHSVSIQWRILGSPCNFSLIYSSDTLGAALCPTFRIDNTTYGCNLQDLQAGTIYNFRIISLDEERTVVLQTDPLPPARFGVSKEKTTSTSLHVWWTPSSGKVTSYEVQLFDENNQKIQGVQIQESTSWNEYTFFNLTAGSKYNIAITAVSGGKRSFSVYTNGSTVPSPVKDIGISTKANSLLISWSHGSGNVERYRLMLMDKGILVHGGVVDKHATSYAFHGLTPGYLYNLTVMTEAAGLQNYRWKLVRTAPMEVSNLKVTNDGSLTSLKVKWQRPPGNVDSYNITLSHKGTIKESRVLAPWITETHFKELVPGRLYQVTVSCVSGELSAQKMAVGRTFPDKVANLEANNNGRMRSLVVSWSPPAGDWEQYRILLFNDSVVLLNITVGKEETQYVMDDTGLVPGRQYEVEVIVESGNLKNSERCQGRTVPLAVLQLRVKHANETSLSIMWQTPVAEWEKYIISLADRDLLLIHKSLSKDAKEFTFTDLVPGRKYMATVTSISGDLKNSSSVKGRTVPAQVTDLHVANQGMTSSLFTNWTQAQGDVEFYQVLLIHENVVIKNESISSETSRYSFHSLKSGSLYSVVVTTVSGGISSRQVVVEGRTVPSSVSGVTVNNSGRNDYLSVSWLLAPGDVDNYEVTLSHDGKVVQSLVIAKSVRECSFSSLTPGRLYTVTITTRSGKYENHSFSQERTVPDKVQGVSVSNSARSDYLRVSWVHATGDFDHYEVTIKNKNNFIQTKSIPKSENECVFVQLVPGRLYSVTVTTKSGQYEANEQGNGRTIPEPVKDLTLRNRSTEDLHVTWSGANGDVDQYEIQLLFNDMKVFPPFHLVNTATEYRFTSLTPGRQYKILVLTISGDVQQSAFIEGFTVPSAVKNIHISPNGATDSLTVNWTPGGGDVDSYTVSAFRHSQKVDSQTIPKHVFEHTFHRLEAGEQYQIMIASVSGSLKNQINVVGRTVPASVQGVIADNAYSSYSLIVSWQKAAGVAERYDILLLTENGILLRNTSEPATTKQHKFEDLTPGKKYKIQILTVSGGLFSKEAQTEGRTVPAAVTDLRITENSTRHLSFRWTASEGELSWYNIFLYNPDGNLQERAQVDPLVQSFSFQNLLQGRMYKMVIVTHSGELSNESFIFGRTVPASVSHLRGSNRNTTDSLWFNWSPASGDFDFYELILYNPNGTKKENWKDKDLTEWRFQGLVPGRKYVLWVVTHSGDLSNKVTAESRTAPSPPSLMSFADIANTSLAITWKGPPDWTDYNDFELQWLPRDALTVFNPYNNRKSEGRIVYGLRPGRSYQFNVKTVSGDSWKTYSKPIFGSVRTKPDKIQNLHCRPQNSTAIACSWIPPDSDFDGYSIECRKMDTQEVEFSRKLEKEKSLLNIMMLVPHKRYLVSIKVQSAGMTSEVVEDSTITMIDRPPPPPPHIRVNEKDVLISKSSINFTVNCSWFSDTNGAVKYFTVVVREADGNDELKPEQQHPLPSYLEYRHNASIRVYQTNYFASKCAENPNSNSKSFNIKLGAEMESLGGKCDPTQQKFCDGPLKPHTAYRISIRAFTQLFDEDLKEFTKPLYSDTFFSLPITTESEPLFGAIE

SEQ ID NO: 5 - DNA, 6199 bp, Mus musculus
ggcacgagggcggctgccacggcccttgagcatcgccagccccgagggtagcgcgctgcgcccgcccgcagggcgcgctgagcgctcaacaagtggtacccagaagtgccctggctggcctcccagcgagatgctgaggcatggagccctaacggccttgtggataacactgagcgtcgtgcagactggagtggcagagcaagtgaaatgtaacttcacactgttggagtccagggtctctagcttgtcagcgtctatccagtggaggactttcgcgtcaccctgtaactttagcctcatctacagcagtgatacctcggggcccatgtggtgccatcctattcggatagacaactttacctacggatgtaaccccaaggatttacaagcagggaccgtctataacttcaggattgtttctctggatggagaagagagcactctggtcttacagacagatccgttgcctcctgccaggtttgaagtcaatcgggagaaaacagcatcaaccaccctgcaggtccggtggactccctcttctggaaaagtctcctggtatgaggtgcaattatttgatcataacaatcaaaagatacaagaagtccaagttcaagaaagtaccacctggagccaatatacttttctgaacctcactgagggtaacagttacaaagttgccatcacagctgtttcgggagaaaagcgctcctttccggtgtatatcaatggctctacagtaccatctccagtgaaagatcttggcatttcccccaatcctaattctctcctaatttcctggtctcgtggttctgggaatgtggaacaatacaggctggtgctaatggataaaggggccatcgttcaagacacaaacgtggacaggcgtgatacttcttatgcttttcacgagctgacccctggccacctctacaacctcactattgtcaccatggcctcgggactgcaaaactccaggtggaaactggtgaggaccgctcccatggaagtctcaaatctgaaggtgacaaatgacgggaggttgacctctctaaatgtgaagtggcagaaaccccctggggatgtagattcctacagcattaccctgtctcaccaagggaccatcaaagaatccaaaacattagcacctcctgttactgaaactcaatttaaggacttagtccctggacggctttaccaagtgaccatcagctgcatctctggtgagctctctgctgagaagtcagcagcggggagaacagttccagaaaaagtgaggaatctggtttcctacaacgagatttggatgaagtcctttacagtgaactggacgccccctgctggagattgggagcattatcgtatcgtgctcttcaatgaatccttggtcttgctcaacaccacagtgggaaaggaagaaacgcactatgccttggatggcttggagctcataccaggaagacagtatgagatagaagtcattgttgagagcggaaatctgcggaattccgagcgctgtcaaggcaggacagtacccctggctgtcctccagcttcgcgtcaaacacgctaacgaaacttcactgggcatcacgtggcgggcccctctaggcgaatgggagaaatacatcatttcgttgatggacagagagctcttggtcatccacaagtcactctccaaagatgccaaagaattcacttttacagacctgatgcctggacggaattacaaggctactgtcactagcatgagtggagatttaaaacagtcatcttcaatcaaaggaagaacagtgcctgcccaggtgactgacctgcacgtcaacaaccaagggatgaccagtagtctgttcactaactggacaaaggcactgggagatgtagagttctaccaagttttactgatccatgaaaatgtggttgtcaagaacgagagtgtttccagtgataccagcagatacagcttccgcgccctgaaacccggcagcctctactccgtggtggtgaccacggtgagtggagggatctcctcccggcaggtggtggcggaaggaagaacagtcccgtccagcgtgagtggggtgacagtcaacaattctggccggaatgactacctcagcgtttcctggctgccggcgcctggagaagtggatcactacgtggtgagcctctcccacgagggcaaggtggatcagttcctcatcatcgccaaatctgtcagcgagtgttccttcagctccctcaccccgggccgcctctacaacgtcactgtaaccaccaagagcggcaattatgcaagccactccttcaccgaggaacggacagtgccagacaaggtccagggaatcagtgttagcaactctgccagaagcgactacttaaaggtgtcctgggtgcatgccactggagactttgaccactatgaagtcaccatcaaaaacagagaaagcttcattcaaaccaaaaccatccccaagtcagaaaatgagtgtgaatttattgagctggttcctggacgcctgtacagcgtcactgtcagtacaaagagtggacaatatgaagccagtgaacaggggacagggagaacgatcccagagcctgtgaaggatctcacccttctcaacaggagtacggaggatctccatgtgacttggtcaagagccaatggggatgttgatcagtacgaggtccagctgctcttcaacgacatgaaagtcttccctcatattcaccttgtgaacacagcaactgagtataagttcacggcgctcacgccggggcgccattacaaaatcctcgtcctgaccatcagtggcgatgtccagcagtcagccttcattgaaggcctcccagttcccagcactgtcaaaaacattcacatttctgccaatggagccacggataggctgatggtaacctggagccctggtggcggggatgtggactcctatgtggtgtctgcattcagacaggacgagaaggttgactctcagaccattcccaagcatgcctcggagcacacgttccacaggctggaggccggagccaagtacaggatcgccattgtttctgtcagtgggtccctgagaaaccagatagatgcgctcggacagacagtcccagcgtctgtccagggagtcgtcgcagccaatgcatacagcagtaattccttaacagtaagttggcagaaagcccttggtgtggcagaaagatacgatatcctgcttctaaacgagaatgggcttcttttgagcaacgtgtcagagccagctacggcaagacagcacaaatttgaagatctaacgccaggcaagaaatacaagatgcagatcctgactgtcagcggaggcctcttcagtaaagaatctcaggctgaaggccgaacagtcccagcagctgtcaccaatctgaggatcacagagaactccagtagatacctgtccttcggctggaccgcctcggagggtgaactcagctggtacaacatcttcctctacaacccagacaggactcttcaggagcgagctcaagttgacccgctagtccagagcttctctttccagaacttgctacaaggcagaatgtacaagatggtgattgtcactcacagtggggagctgtccaatgagtcatttatattcggcagaacagttcctgctgccgtgaaccatctcaaaggctcccatcggaacacgacagacagcctgtggttcagctggagcccagcctccggggactttgacttctatgagctgattctttacaatcccaacggcacgaagaaggagaactggaaagaaaaggacgtgacagagtggcgtttccaaggtcttgttcctggaaggaaatacaccctgtatgtggtgactcacagtggggacctcagcaataaagtcacaggggagggcagaacagccccaagtcctccgagtcttttgtcattcgctgatgttgcaaacacctccttggctatcacctggaagggacccccagactggacagattacaatgactttgagctgcagtggttccctggagatgcacttaccatcttcaacccctacagcagcagaaagtcagaaggacgcattgtgtacgggcttcacccagggaggtcctatcaattcagtgtcaagactgtgagcggggactcctggaaaacctacagcaaaccaatttctgggtctgtgaggacaaagccagacaagatacaaaacctgcattgccgcccccagaactccacggccattgcctgctcttggatacctcctgactccgactttgatggctacagcattgagtgccgaaaaatggatacccaagaaatcgagttttccagaaagctggagaaagaaaaatcactgctcaacatcatgatgttagtacctcataagaggtacctggtgtccatcaaggtgcagtcggccggcatgaccagtgaggtggttgaagatagcaccatcaccatgatagaccgcccgcctcaaccgcctccacacatccgtgtgaatgaaaaggatgtgctaatcagcaaatcttccatcaactttactgtcaactgcagctggttcagcgacaccaacggagcggttaaatactttgctgtggtggtgagagaggccgacagcatggatgagttgaagccagaacagcagcaccctctcccttcctacctggagtacagacacaacgcctccatccgagtctaccagaccaattattttgccagcaaatgtgctgaaagtcccgacagcagttctaaaagtttcaacattaagcttggagcagagatggacagcctcggtggcaaatgtgatcccagtcagcagaaattctgtgatggaccgctgaagccacacaccgcctacagaatcagcatccgggcttttacacagctatttgacgaggacttgaaagagttcaccaaacctctctactcggatacgttcttctctatgcccatcaccacagagtcagagcccttgtttggagttattgaaggtgtgagtgctggcctgtttctaattggcatgctggtggcccttgttgccttcttcatctgcagacagaaagctagccacagcagggaaaggccatctgcccggctcagcattcgtagggaccggcctttgtctgtccatctgaatctgggccagaaaggcaaccggaaaacttcttgccccataaagatcaatcagtttgaagggcatttcatgaagctgcaggcagactccaactaccttctatccaaggaatatgaggacttaaaagacgtgggtagaagccagtcatgtgacattgccctcttgcctgagaatcgagggaaaaatcgatacaacaacatattgccttatgatgcctcaagagtgaagctctcgaatgtcgatgacgacccttgctctgactacatcaacgccagctacatccccggtaacaacttcagacgagaatacatcgccactcagggaccgcttccaggcaccaaggatgacttctggaagatggcgtgggagcagaacgttcacaacatcgtcatggtgacccagtgtgttgaaaagggccgagtgaagtgtgaccattactggccagcagaccaggaccccctctactacggtgatctcatcctacagatggtctcggagtccgtgctccccgagtggaccatcagggagtttaagatatgcagtgaagaacagttggatgcacacagactcatccgtcactttcactacacggtgtggccagaccatggggtcccagagaccacccagtccctgatccaatttgtgaggacagtcagggactacatcaacagaagccccggggctgggcccaccgtagtgcactgcagcgctggtgtgggcagaacagggacgttcgttgccctggaccggatcctccagcagttggactctaaggactccgtggacatttatggggcagtgcatgacctaagactccacagggttcacatggtccagaccgagtgtcaatatgtgtatctgcatcagtgtgtaagagacgtcctcagagcaaagaaactgcggaacgagcaagagaaccccctgtttccgatttatgagaatgtgaatccagagtatcacagagatgcaatctactcgagacattaagaattcacctgaagatcccctggataaaagcgtttcactgtgtgactttaaaaaaaaaaaaaaaaaaaaaaa

SEQ ID NO: 6 - protein, 1998 aa, Mus musculus
MLRHGALTALWITLSVVQTGVAEQVKCNFTLLESRVSSLSASIQWRTFASPCNFSLIYSSDTSGPMWCHPIRIDNFTYGCNPKDLQAGTVYNFRIVSLDGEESTLVLQTDPLPPARFEVNREKTASTTLQVRWTPSSGKVSWYEVQLFDHNNQKIQEVQVQESTTWSQYTFLNLTEGNSYKVAITAVSGEKRSFPVYINGSTVPSPVKDLGISPNPNSLLISWSRGSGNVEQYRLVLMDKGAIVQDTNVDRRDTSYAFHELTPGHLYNLTIVTMASGLQNSRWKLVRTAPMEVSNLKVTNDGRLTSLNVKWQKPPGDVDSYSITLSHQGTIKESKTLAPPVTETQFKDLVPGRLYQVTISCISGELSAEKSAAGRTVPEKVRNLVSYNEIWMKSFTVNWTPPAGDWEHYRIVLFNESLVLLNTTVGKEETHYALDGLELIPGRQYEIEVIVESGNLRNSERCQGRTVPLAVLQLRVKHANETSLGITWRAPLGEWEKYIISLMDRELLVIHKSLSKDAKEFTFTDLMPGRNYKATVTSMSGDLKQSSSIKGRTVPAQVTDLHVNNQGMTSSLFTNWTKALGDVEFYQVLLIHENVVVKNESVSSDTSRYSFRALKPGSLYSVVVTTVSGGISSRQVVAEGRTVPSSVSGVTVNNSGRNDYLSVSWLPAPGEVDHYVVSLSHEGKVDQFLIIAKSVSECSFSSLTPGRLYNVTVTTKSGNYASHSFTEERTVPDKVQGISVSNSARSDYLKVSWVHATGDFDHYEVTIKNRESFIQTKTIPKSENECEFIELVPGRLYSVTVSTKSGQYEASEQGTGRTIPEPVKDLTLLNRSTEDLHVTWSRANGDVDQYEVQLLFNDMKVFPHIHLVNTATEYKFTALTPGRHYKILVLTISGDVQQSAFIEGLPVPSTVKNIHISANGATDRLMVTWSPGGGDVDSYVVSAFRQDEKVDSQTIPKHASEHTFHRLEAGAKYRIAIVSVSGSLRNQIDALGQTVPASVQGVVAANAYSSNSLTVSWQKALGVAERYDILLLNENGLLLSNVSEPATARQHKFEDLTPGKKYKMQILTVSGGLFSKESQAEGRTVPAAVTNLRITENSSRYLSFGWTASEGELSWYNIFLYNPDRTLQERAQVDPLVQSFSFQNLLQGRMYKMVIVTHSGELSNESFIFGRTVPAAVNHLKGSHRNTTDSLWFSWSPASGDFDFYELILYNPNGTKKENWKEKDVTEWRFQGLVPGRKYTLYVVTHSGDLSNKVTGEGRTAPSPPSLLSFADVANTSLAITWKGPPDWTDYNDFELQWFPGDALTIFNPYSSRKSEGRIVYGLHPGRSYQFSVKTVSGDSWKTYSKPISGSVRTKPDKIQNLHCRPQNSTAIACSWIPPDSDFDGYSIECRKMDTQEIEFSRKLEKEKSLLNIMMLVPHKRYLVSIKVQSAGMTSEVVEDSTITMIDRPPQPPPHIRVNEKDVLISKSSINFTVNCSWFSDTNGAVKYFAVVVREADSMDELKPEQQHPLPSYLEYRHNASIRVYQTNYFASKCAESPDSSSKSFNIKLGAEMDSLGGKCDPSQQKFCDGPLKPHTAYRISIRAFTQLFDEDLKEFTKPLYSDTFFSMPITTESEPLFGVIEGVSAGLFLIGMLVALVAFFICRQKASHSRERPSARLSIRRDRPLSVHLNLGQKGNRKTSCPIKINQFEGHFMKLQADSNYLLSKEYEDLKDVGRSQSCDIALLPENRGKNRYNNILPYDASRVKLSNVDDDPCSDYINASYIPGNNFRREYIATQGPLPGTKDDFWKMAWEQNVHNIVMVTQCVEKGRVKCDHYWPADQDPLYYGDLILQMVSESVLPEWTIREFKICSEEQLDAHRLIRHFHYTVWPDHGVPETTQSLIQFVRTVRDYINRSPGAGPTVVHCSAGVGRTGTFVALDRILQQLDSKDSVDIYGAVHDLRLHRVHMVQTECQYVYLHQCVRDVLRAKKLRNEQENPLFPIYENVNPEYHRDAIYSRH

SEQ ID NO: 7 - protein, 1619 aa, Mus musculus
MLRHGALTALWITLSVVQTGVAEQVKCNFTLLESRVSSLSASIQWRTFASPCNFSLIYSSDTSGPMWCHPIRIDNFTYGCNPKDLQAGTVYNFRIVSLDGEESTLVLQTDPLPPARFEVNREKTASTTLQVRWTPSSGKVSWYEVQLFDHNNQKIQEVQVQESTTWSQYTFLNLTEGNSYKVAITAVSGEKRSFPVYINGSTVPSPVKDLGISPNPNSLLISWSRGSGNVEQYRLVLMDKGAIVQDTNVDRRDTSYAFHELTPGHLYNLTIVTMASGLQNSRWKLVRTAPMEVSNLKVTNDGRLTSLNVKWQKPPGDVDSYSITLSHQGTIKESKTLAPPVTETQFKDLVPGRLYQVTISCISGELSAEKSAAGRTVPEKVRNLVSYNEIWMKSFTVNWTPPAGDWEHYRIVLFNESLVLLNTTVGKEETHYALDGLELIPGRQYEIEVIVESGNLRNSERCQGRTVPLAVLQLRVKHANETSLGITWRAPLGEWEKYIISLMDRELLVIHKSLSKDAKEFTFTDLMPGRNYKATVTSMSGDLKQSSSIKGRTVPAQVTDLHVNNQGMTSSLFTNWTKALGDVEFYQVLLIHENVVVKNESVSSDTSRYSFRALKPGSLYSVVVTTVSGGISSRQVVAEGRTVPSSVSGVTVNNSGRNDYLSVSWLPAPGEVDHYVVSLSHEGKVDQFLIIAKSVSECSFSSLTPGRLYNVTVTTKSGNYASHSFTEERTVPDKVQGISVSNSARSDYLKVSWVHATGDFDHYEVTIKNRESFIQTKTIPKSENECEFIELVPGRLYSVTVSTKSGQYEASEQGTGRTIPEPVKDLTLLNRSTEDLHVTWSRANGDVDQYEVQLLFNDMKVFPHIHLVNTATEYKFTALTPGRHYKILVLTISGDVQQSAFIEGLPVPSTVKNIHISANGATDRLMVTWSPGGGDVDSYVVSAFRQDEKVDSQTIPKHASEHTFHRLEAGAKYRIAIVSVSGSLRNQIDALGQTVPASVQGVVAANAYSSNSLTVSWQKALGVAERYDILLLNENGLLLSNVSEPATARQHKFEDLTPGKKYKMQILTVSGGLFSKESQAEGRTVPAAVTNLRITENSSRYLSFGWTASEGELSWYNIFLYNPDRTLQERAQVDPLVQSFSFQNLLQGRMYKMVIVTHSGELSNESFIFGRTVPAAVNHLKGSHRNTTDSLWFSWSPASGDFDFYELILYNPNGTKKENWKEKDVTEWRFQGLVPGRKYTLYVVTHSGDLSNKVTGEGRTAPSPPSLLSFADVANTSLAITWKGPPDWTDYNDFELQWFPGDALTIFNPYSSRKSEGRIVYGLHPGRSYQFSVKTVSGDSWKTYSKPISGSVRTKPDKIQNLHCRPQNSTAIACSWIPPDSDFDGYSIECRKMDTQEIEFSRKLEKEKSLLNIMMLVPHKRYLVSIKVQSAGMTSEVVEDSTITMIDRPPQPPPHIRVNEKDVLISKSSINFTVNCSWFSDTNGAVKYFAVVVREADSMDELKPEQQHPLPSYLEYRHNASIRVYQTNYFASKCAESPDSSSKSFNIKLGAEMDSLGGKCDPSQQKFCDGPLKPHTAYRISIRAFTQLFDEDLKEFTKPLYSDTFFSMPITTESEPLFG